European Patent Application EP 4 393 942 A1, published July 3, 2024. Title: TCR, Polypeptide, Expression vector, Host cell, Pharmaceutical Composition and Method for Obtaining TCR. Applicant: Keshihua (Nanjing) Biotechnology Co., Ltd. The sequence listing filed with the application follows.

SEQUENCE LISTING (255 sequences)

SEQ ID NO: 1 - protein, 145 aa, synthetic construct
MVLKFSVSILWIQLAWVSTQLLEQSPQFLSIQEGENLTVYCNSSSVFSSLQWYRQEPGEGPVLLVTVVTGGEVKKLKRLTFQFGDARKDSSLHITAAQPGDTGLYLCAGDGSGNTGKLIFGQGTTLQVKPDIQNPDPAVYQLRDX

SEQ ID NO: 2 - protein, 150 aa, synthetic construct
MLLEHLLIILWMQLTWVSGQQLNQSPQSMFIQEGEDVSMNCTSSSIFNTWLWYKQDPGEGPVLLIALYKAGELTSNGRLTAQFGITRKDSFLNISASIPSDVGIYFCAGAGGFLNSGGSKYKLTFGKGTLLTVNPNIQNPDPAVYQLRDX

SEQ ID NO: 3 - protein, 149 aa, synthetic construct
MTRVSLLWAVVVSTCLESGMAQTVTQSQPEMSVQEAETVTLSCTYDTSESNYYLFWYKQPPSRQMILVIRQEAYKQQNATENRFSVNFQKAAKSFSLKISDSQLGDTAMYFCAFMKGSNYKLTFGKGTLLTVNPNIQNPDPAVYQLRDX

SEQ ID NO: 4 - protein, 135 aa, synthetic construct
MTRVSLLWAVVVSTCLESGMAQTVTQSQPEMSVQEAETVTLSCTYDTSENNYYLFWYKQPPSRQMILVIRQEAYKQQNATENRFSVNFQKAAKSFSLKISDSQLGDTAMYFCATHSGAGSYQLTFGKGTKLSVIP

SEQ ID NO: 5 - protein, 144 aa, synthetic construct
MLLITSMLVLWMQLSQVNGQQVMQIPQYQHVQEGEDFTTYCNSSTTLSNIQWYKQRPGGHPVFLIQLVKSGEVKKQKRLTFQFGEAKKNSSLHITATQTTDVGTYFCAGNVGGTGKLIFGQGTTLQVKPDIQNPDPAVYQLRDX

SEQ ID NO: 6 - protein, 141 aa, synthetic construct
MRLVARVTVFLTFGTIIDAKTTQPPSMDCAEGRAANLPCNHSTISGNEYVYWYRQIHSQGPQYIIHGLKNNETNEMASLIITEDRKSSTLILPHATLRDTAVYYCQRRDTGNQFYFGTGTSLTVIPNIQNPDPAVYQLRDX

SEQ ID NO: 7 - protein, 151 aa, synthetic construct
MLTASLLRAVIASICVVSSMAQKVTQAQTEISVVEKEDVTLDCVYETRDTTYYLFWYKQPPSGELVFLIRRNSFDEQNEISGRYSWNFQKSTSSFNFTITASQVVDSAVYFCALSEIKNQGGKLIFGQGTELSVKPNIQNPDPAVYQLRDX

SEQ ID NO: 8 - protein, 143 aa, synthetic construct
METLLGLLILWLQLQWVSSKQEVTQIPAALSVPEGENLVLNCSFTDSAIYNLQWFRQDPGKGLTSLLLIQSSQREQTSGRLNASLDKSSGRSTLYIAASQPGDSATYLCAVRPGELSFGAGTTVTVRANIQNPDPAVYQLRDX

SEQ ID NO: 9 - protein, 149 aa, synthetic construct
MASAPISMLAMLFTLSGLRAQSVAQPEDQVNVAEGNPLTVKCTYSVSGNPYLFWYVQYPNRGLQFLLKYITGDNLVKGSYGFEAEFNKSQTSFHLKKPSALVSDSALYFCAVRDEGGATNKLIFGTGTLLAVQPNIQNPDPAVYQLRDX

SEQ ID NO: 10 - protein, 149 aa, synthetic construct
MLLLLIPVLGMIFALRDARAQSVSQHNHHVILSEAASLELGCNYSYGGTVNLFWYVQYPGQHLQLLLKYFSGDPLVKGIKGFEAEFIKSKFSFNLRKPSVQWSDTAEYFCAVNAGGGSQGNLIFGKGTKLSVKPNIQNPDPAVYQLRDX

SEQ ID NO: 11 - protein, 146 aa, synthetic construct
MLLLLVPAFQVIFTLGGTRAQSVTQLDSQVPVFEEAPVELRCNYSSSVSVYLFWYVQYPNQGLQLLLKYLSGSTLVKGINGFEAEFNKSQTSFHLRKPSVHISDTAEYFCAVSGSGDKLIFGTGTRLQVFPNIQNPDPAVYQLRDX

SEQ ID NO: 12 - protein, 164 aa, synthetic construct
DQKRRLLTLQQGPVSMACPGFLWALVISTCLEFSMAQTVTQSQPEMSVQEAETVTLSCTYDTSESDYYLFWYKQPPSRQMILVIRQEAYKQQNATENRFSVNFQKAAKSFSLKISDSQLGDAAMYFCASFSGGYQKVTFGTGTKLQVIPNIQNPDPAVYQLRDX

SEQ ID NO: 13 - protein, 150 aa, synthetic construct
METVLQVLLGILGFQAAWVSSQELEQSPQSLIVQEGKNLTINCTSSKTLYGLYWYKQKYGEGLIFLMMLQKGGEEKSHEKITAKLDEKKQQSSLHITASQPSHAGIYLCGAGRPNSGGSNYKLTFGKGTLLTVNPNIQNPDPAVYQLRDX

SEQ ID NO: 14 - protein, 145 aa, synthetic construct
MTSIRAVFIFLWLQLDLVNGENVEQHPSTLSVQEGDSAVIKCTYSDSASNYFPWYKQELGKRPQLIIDIRSNVGEKKDQRIAVTLNKTAKHFSLHITETQPEDSAVYFCAAGGRDDKIIFGKGTRLHILPNIQNPDPAVYQLRDX

SEQ ID NO: 15 - protein, 144 aa, synthetic construct
MWGVFLLYVSMKMGGTTGQNIDQPTEMTATEGAIVQINCTYQTSGFNGLFWYQQHAGEAPTFLSYNVLDGLEEKGRFSSFLSRSKGYSYLLLKELQMKDSASYLCAVRPSNQAGTALIFGKGTTLSVSSNIQNPDPAVYQLRDX

SEQ ID NO: 16 - protein, 147 aa, synthetic construct
MEKNPLAAPLLILWFHLDCVSSILNVEQSPQSLHVQEGDSTNFTCSFPSSNFYALHWYRWETAKSPEALFVMTLNGDEKKKGRISATLNTKEGYSYLYIKGSQPEDSATYLCASLYFNKFYFGSGTKLNVKPNIQNPDPAVYQLRDX

SEQ ID NO: 17 - protein, 145 aa, synthetic construct
MTSIRAVFIFLWLQLDLVNGENVEQHPSTLSVQEGDSAVIKCTYSDSASNYFPWYKQELGKRPQLIIDIRSNVGEKKDQRIAVTLNKTAKHFSLHITETQPEDSAVYFCAAIGFGNVLHCGSGTQVIVLPHIQNPDPAVYQLRDX

SEQ ID NO: 18 - protein, 144 aa, synthetic construct
MLLITSMLVLWMQLSQVNGQQVMQIPQYQHVQEGEDFTTYCNSSTTLSNIQWYKQRPGGHPVFLIQLVKSGEVKKQKRLTFQFGEAKKNSSLHITATQTTDVGTYFCAGAPSNDYKLSFGAGTTVTVRANIQNPDPAVYQLRDX

SEQ ID NO: 19 - protein, 142 aa, synthetic construct
MVLKFSVSILWIQLAWVSTQLLEQSPQFLSIQEGENLTVYCNSSSVFSSLQWYRQEPGEGPVLLVTVVTGGEVKKLKRLTFQFGDARKDSSLHITAAQPGDTGLYLCAGADNNDMRFGAGTRLTVKPNIQNPDPAVYQLRDX

SEQ ID NO: 20 - protein, 144 aa, synthetic construct
MLLITSMLVLWMQLSQVNGQQVMQIPQYQHVQEGEDFTTYCNSSTTLSNIQWYKQRPGGHPVFLIQLVKSGEVKKQKRLTFQFGEAKKNSSLHITATQTTDVGTYFCGTSNFGNEKLTFGTGTRLTIIPNIQNPDPAVYQLRDX

SEQ ID NO: 21 - protein, 149 aa, synthetic construct
MAGIRALFMYLWLQLDWVSRGESVGLHLPTLSVQEGDNSIINCAYSNSASDYFIWYKQESGKGPQFIIDIRSNMDKRQGQRVTVLLNKTVKHLSLQIAATQPGDSAVYFCAENDSGGGADGLTFGKGTHLIIQPYIQNPDPAVYQLRDX

SEQ ID NO: 22 - protein, 146 aa, synthetic construct
MTSIRAVFIFLWLQLDLVNGENVEQHPSTLSVQEGDSAVIKCTYSDSASNYFPWYKQELGKGPQLIIDIRSNVGEKKDQRIAVTLNKTAKHFSLHITETQPEDSAVYFCAAMRGGADGLTFGKGTHLIIQPYIQNPDPAVYQLRDX

SEQ ID NO: 23 - protein, 145 aa, synthetic construct
METLLGLLILWLQLQWVSSKQEVTQIPAALSVPEGENLVLNCSFTDSAIYNLQWFRQDPGKGLTSLLLIQSSQREQTSGRLNASLDKSSGRSTLYIAASQPGDSATYLCAVTGGADGLTFGKGTHLIIQPYIQNPDPAVYQLRDX

SEQ ID NO: 24 - protein, 139 aa, synthetic construct
MWGAFLLYVSMKMGGTAGQSLEQPSEVTAVEGAIVQINCTYQTSGFYGLSWYQQHDGGAPTFLSYNALDGLEETGRFSSFLSRSDSYGYLLLQELQMKDSASYFCADQGGKLIFGQGTELSVKPNIQNPDPAVYQLRDX

SEQ ID NO: 25 - protein, 147 aa, synthetic construct
MMKSLRVLLVILWLQLSWVWSQQKEVEQDPGPLSVPEGAIVSLNCTYSNSAFQYFMWYRQYSRKGPELLMYTYSSGNKEDGRFTAQVDKSSKYISLFIRDSQPSDSATYLCAMKTSYDKVIFGPGTSLSVIPNIQNPDPAVYQLRDX

SEQ ID NO: 26 - protein, 144 aa, synthetic construct
MVLKFSVSILWIQLAWVSTQLLEQSPQFLSIQEGENLTVYCNSSSVFSSLQWYRQEPGEGPVLLVTVVTGGEVKKLKRLTFQFGDARKDSSLHITAAQPGDTGLYLCAASGGSNYKLTFGKGTLLTVNPNIQNPDPAVYQLRDX

SEQ ID NO: 27 - protein, 147 aa, synthetic construct
MISLRVLLVILWLQLSWVWSQRKEVEQDPGPFNVPEGATVAFNCTYSNSASQSFFWYRQDCRKEPKLLMSVYSSGNEDGRFTAQLNRASQYISLLIRDSKLSDSATYLCAVNPSRGYSTLTFGKGTMLLVSPDIQNPDPAVYQLRDX

SEQ ID NO: 28 - protein, 144 aa, synthetic construct
METLLGLLILWLQLQWVSSKQEVTQIPAALSVPEGENLVLNCSFTDSAIYNLQWFRQDPGKGLTSLLLIQSSQREQTSGRLNASLDKSSGRSTLYIAASQPGDSATYLCAVYGNNRLAFGKGNQVVVIPNIQNPDPAVYQLRDX

SEQ ID NO: 29 - protein, 146 aa, synthetic construct
MLLELIPLLGIHFVLRTARAQSVTQPDIHITVSEGASLELRCNYSYGATPYLFWYVQSPGQGLQLLLKYFSGDTLVQGIKGFEAEFKRSQSSFNLRKPSVHWSDAAEYFCAVGYGNNRLAFGKGNQVVVIPNIQNPDPAVYQLRDX

SEQ ID NO: 30 - protein, 147 aa, synthetic construct
MTSIRAVFIFLWLQLDLVNGENVEQHPSTLSVQEGDSAVIKCTYSDSASNYFPWYKQELGKRPQLIIDIRSNVGEKKDQRIAVTLNKTAKHFSLHITETQPEDSAVYFCAAGPSNTGNQFYFGTGTSLTVIPNIQNPDPAVYQLRDX

SEQ ID NO: 31 - protein, 160 aa, synthetic construct
MGTSLLCWMALCLLGADHADTGVSQDPRHKITKRGQNVTFRCDPISEHNRLYWYRQTLGQGPEFLTYFQNEAQLEKSRLLSDRFSAERPKGSFSTLEIQRTEQGDSAMYLCASSHNGLGQGEDLLSGANVLTFGAGSRLTVLEDLKNVFPPEVAVFEPSX

SEQ ID NO: 32 - protein, 149 aa, synthetic construct
MSNQVLCCVVLCFLGANTVDGGITQSPKYLFRKEGQNVTLSCEQNLNHDAMYWYRQDPGQGLRLIYYSQIVNDFQKGDIAEGYSVSREKKESFPLTVTSAQKNPTAFYLCASSIPGGYGYTFGSGTRLTVVEDLNKVFPPEVAVFEPSX

SEQ ID NO: 33 - protein, 154 aa, synthetic construct
MGTSLLCWMALCLLGADHADTGVSQDPRHKITKRGQNVTFRCDPISEHNRLYWYRQTLGQGPEFLTYFQNEAQLEKSRLLSDRFSAERPKGSFSTLEIQRTEQGDSAMYLCASSPVNPAVSYNEQFFGPGTRLTVLEDLKNVFPPEVAVFEPSX

SEQ ID NO: 34 - protein, 132 aa, synthetic construct
MGTSLLCWMALCLLGADHADTGVSQNPRHKITKRGQNVTFRCDPISEHNRLYWYRQTLGQGPEFLTYFQNEAQLEKSRLLSDRFSAERPKGSFSTLEIQRTEQGDSAMYLCASSAPGYNEQFFGPGTRLTVL

SEQ ID NO: 35 - protein, 151 aa, synthetic construct
MLLLLLLLGPGSGLGAVVSQHPSWVICKSGTSVKIECRSLDFQATTMFWYRQFPKQSLMLMATSNEGSKATYEQGVEKDKFLINHASLTLSTLTVTSAHPEDSSFYICSARFIPTGLGENTIYFGEGSWLTVVEDLNKVFPPEVAVFEPSX

SEQ ID NO: 36 - protein, 152 aa, synthetic construct
MGPGLLCWVLLCLLGAGPVDAGVTQSPTHLIKTRGQHVTLRCSPISGHKSVSWYQQVLGQGPQFIFQYYEKEERGRGNFPDRFSARQFPNYSSELNVNALLLGDSALYLCASSLTAGAYTGELFFGEGSRLTVLEDLKNVFPPEVAVFEPSX

SEQ ID NO: 37 - protein, 154 aa, synthetic construct
MGCRLLCCAVLCLLGAVPIDTEVTQTPKHLVMGMTNKKSLKCEQHMGHRAMYWYKQKAKKPPELMFVYSYEKLSINESVPSRFSPECPNSSLLNLHLHALQPEDSALYLCASSQGVERQGPRNEQFFGPGTRLTVLEDLKNVFPPEVAVFEPSX

SEQ ID NO: 38 - protein, 150 aa, synthetic construct
MGPQLLGYVVLCLLGAGPLEAQVTQNPRYLITVTGKKLTVTCSQNMNHEYMSWYRQDPGLGLRQIYYSMNVEVTDKGDVPEGYKVSRKEKRNFPLILESPSPNQTSLYFCASSSSGRNNEQFFGPGTRLTVLEDLKNVFPPEVAVFEPSX

SEQ ID NO: 39 - protein, 149 aa, synthetic construct
MSNQVLCCVVLCFLGANTVDGGITQSPKYLFRKEGQNVTLSCEQNLNHDAMYWYRQDPGQGLRLIYYSQIVNDFQKGDIAEGYSVSREKKESFPLTVTSAQKNPTAFYLCASSIAHGDEQYFGPGTRLTVTEDLKNVFPPEVAVFEPSX

SEQ ID NO: 40 - protein, 151 aa, synthetic construct
MGCRLLCCAVLCLLGAVPIDTEVTQTPKHLVMGMTNKKSLKCEQHMGHRAMYWYKQKAKKPPELMFVYSYEKLSINESVPSRFSPECPNSSLLNLHLHALQPEDSALYLCASQDYLNSYNEQFFGPGTRLTVLEDLKNVFPPEVAVFEPSX

SEQ ID NO: 41 - protein, 154 aa, synthetic construct
MGTSLLCWMALCLLGADHADTGVSQDPRHKITKRGQNVTFRCDPISEHNRLYWYRQTLGQGPEFLTYFQNEAQLEKSRLLSDRFSAERPKGSFSTLEIQRTEQGDSAMYLCASSLARQGVDQETQYFGPGTRLLVLEDLKNVFPPEVAVFEPSX

SEQ ID NO: 42 - protein, 161 aa, synthetic construct
RPHLRPEASMGCRLLCCAVLCLLGAVPIDTEVTQTPKHLVMGMTNKKSLKCEQHMGHRAMYWYKQKAKKPPELMFVYSYEKLSINESVPSRFSPECPNSSLLNLHLHALQPEDSALYLCASSQDKYRGNEKLFFGSGTQLSVLEDLNKVFPPEVAVFEPSX

SEQ ID NO: 43 - protein, 149 aa, synthetic construct
MGCRLLCCAVLCLLGAVPMETGVTQTPRHLVMGMTNKKSLKCEQHLGHNAMYWYKQSAKKPLELMFVYSLEERVENNSVPSRFSPECPNSSHLFLHLHTLQPEDSALYLCASSQDRADTQYFGPGTRLTVLEDLKNVFPPEVAVFEPSX

SEQ ID NO: 44 - protein, 150 aa, synthetic construct
MGPQLLGYVVLCLLGAGPLEAQVTQNPRYLITVTGKKLTVTCSQNMNHEYMSWYRQDPGLGLRQIYYSMNVEVTDKGDVPEGYKVSRKEKRNFPLILESPSPNQTSLYFCASSLGGSRLEQYFGPGTRLTVTEDLKNVFPPEVAVFEPSX

SEQ ID NO: 45 - protein, 152 aa, synthetic construct
MGCRLLCCAVLCLLGAVPIDTEVTQTPKHLVMGMTNKKSLKCEQHMGHRAMYWYKQKAKKPPELMFVYSYEKLSINESVPSRFSPECPNSSLLNLHLHALQPEDSALYLCASSPLDRGLSGELFFGEGSRLTVLEDLKNVFPPEVAVFEPSX

SEQ ID NO: 46 - protein, 152 aa, synthetic construct
MGPQLLGYVVLCLLGAGPLEAQVTQNPRYLITVTGKKLTVTCSQNMNHEYMSWYRQDPGLGLRQIYYSMNVEVTDKGDVPEGYKVSRKEKRNFPLILESPSPNQTSLYFCASSLSFGSGANVLTFGAGSRLTVLEDLKNVFPPEVAVFEPSX

SEQ ID NO: 47 - protein, 150 aa, synthetic construct
MSLGLLCCGAFSLLWAGPVNAGVTQTPKFRVLKTGQSMTLLCAQDMNHEYMYWYRQDPGMGLRLIHYSVGEGTTAKGEVPDGYNVSRLKKQNFLLGLESAAPSQTSVYFCASSYTSNTGELFFGEGSRLTVLEDLKNVFPPEVAVFEPSX

SEQ ID NO: 48 - protein, 148 aa, synthetic construct
MLLLLLLLGPGSGLGAVVSQHPSWVICKSGTSVKIECRSLDFQATTMFWYRQFPKQSLMLMATSNEGSKATYEQGVEKDKFLINHASLTLSTLTVTSAHPEDSSFYICSARGYGQGPEQYFGPGTRLTVTEDLKNVFPPEVAVFEPSX

SEQ ID NO: 49 - protein, 152 aa, synthetic construct
MGPRLLFWALLCLLGTGPVEAGVTQSPTHLIKTRGQQATLRCSPISGHTSVYWYQQALGLGLQFLLWYDEGEERNRGNFPPRFSGRQFPNYSSELNVNALELEDSALYLCASSPGTPFSYNEQFFGPGTRLTVLEDLKNVFPPEVAVFEPSX

SEQ ID NO: 50 - protein, 150 aa, synthetic construct
MGPGLLCWALLCLLGAGLVDAGVTQSPTHLIKTRGQQVTLRCSPKSGHDTVSWYQQALGQGPQFIFQYYEEEERQRGNFPDRFSGHQFPNYSSELNVNALLLGDSALYLCASSFAVYGGELFFGEGSRLTVLEDLKNVFPPEVAVFEPSX

SEQ ID NO: 51 - protein, 151 aa, synthetic construct
MGFRLLCCVAFCLLGAGPVDSGVTQTPKHLITATGQRVTLRCSPRSGDLSVYWYQQSLDQGLQFLIQYYNGEERAKGNILERFSAQQFPDLHSELNLSSLELGDSALYFCASSTLAGTYNEQFFGPGTRLTVLEDLKNVFPPEVAVFEPSX

SEQ ID NO: 52 - protein, 151 aa, synthetic construct
MGTRLLFWVAFCLLGADHTGAGVSQSPSNKVTEKGKDVELRCDPISGHTALYWYRQSLGQGLEFLIYFQGNSAPDKSGLPSDRFSAERTGGSVSTLTIQRTQQEDSAVYLCASSLGPPGGEQFFGPGTRLTVLEDLKNVFPPEVAVFEPSX

SEQ ID NO: 53 - protein, 149 aa, synthetic construct
MSIGLLCCAALSLLWAGPVNAGVTQTPKFQVLKTGQSMTLQCAQDMNHEYMSWYRQDPGMGLRLIHYSVGAGITDQGEVPNGYNVSRSTTEDFPLRLLSAAPSQTSVYFCASSYSNAGELFFGEGSRLTVLEDLKNVFPPEVAVFEPSX

SEQ ID NO: 54 - protein, 151 aa, synthetic construct
MRIRLLCCVAFSLLWAGPVIAGITQAPTSQILAAGRRMTLRCTQDMRHNAMYWYRQDLGLGLRLIHYSNTAGTTGKGEVPDGYSVSRANTDDFPLTLASAVPSQTSVYFCASSLGLAGDDEQFFGPGTRLTVLEDLKNVFPPEVAVFEPSX

SEQ ID NO: 55 - protein, 147 aa, synthetic construct
MTIRLLCYMGFYFLGAGLMEADIYQTPRYLVIGTGKKITLECSQTMGHDKMYWYQQDPGMELHLIHYSYGVNSTEKGDLSSESTVSRIRTEHFPLTLESARPSHTSQYLCASSRGDEQFFGPGTRLTVLEDLKNVFPPEVAVFEPSX

SEQ ID NO: 56 - protein, 151 aa, synthetic construct
MGIRLLCRVAFCFLAVGLVDVKVTQSSRYLVKRTGEKVFLECVQDMDHENMFWYRQDPGLGLRLIYFSYDVKMKEKGDIPEGYSVSREKKERFSLILESASTNQTSMYLCASIGETGFVETQYFGPGTRLLVLEDLKNVFPPEVAVFEPSX

SEQ ID NO: 57 - protein, 150 aa, synthetic construct
MGPQLLGYVVLCLLGAGPLEAQVTQNPRYLITVTGKKLTVTCSQNMNHEYMSWYRQDPGLGLRQIYYSMNVEVTDKGDVPEGYKVSRKEKRNFPLILESPSPNQTSLYFCASSETGIRDGYTFGSGTRLTVVEDLNKVFPPEVAVFEPSX

SEQ ID NO: 58 - protein, 153 aa, synthetic construct
MASLLFFCGAFYLLGTGSMDADVTQTPRNRITKTGKRIMLECSQTKGHDRMYWYRQDPGLGLRLIYYSFDVKDINKGEISDGYSVSRQAQAKFSLSLESAIPNQTALYFCATSDPSDRVGQETQYFGPGTRLLVLEDLKNVFPPEVAVFEPSX

SEQ ID NO: 59 - protein, 149 aa, synthetic construct
MGSRLLCWVLLCLLGAGPVKAGVTQTPRYLIKTRGQQVTLSCSPISGHRSVSWYQQTPGQGLQFLFEYFSETQRNKGNFPGRFSGRQFSNSRSEMNVSTLELGDSALYLCASSLEGSREQYFGPGTRLTVTEDLKNVFPPEVAVFEPSX

SEQ ID NO: 60 - protein, 153 aa, synthetic construct
MGCRLLCCAVLCLLGAVPIDTEVTQTPKHLVMGMTNKKSLKCEQHMGHRAMYWYKQKAKKPPELMFVYSYEKLSINESVPSRFSPECPNSSLLNLHLHALQPEDSALYLCASSLHIAGGISDTQYFGPGTRLTVLEDLKNVFPPEVAVFEPSX

SEQ ID NO: 61 - protein, 5 aa, synthetic construct
SVFSS

SEQ ID NO: 62 - protein, 5 aa, synthetic construct
SIFNT

SEQ ID NO: 63 - protein, 7 aa, synthetic construct
TSESNYY

SEQ ID NO: 64 - protein, 7 aa, synthetic construct
TSENNYY

SEQ ID NO: 65 - protein, 5 aa, synthetic construct
TTLSN

SEQ ID NO: 66 - protein, 7 aa, synthetic construct
TISGNEY

SEQ ID NO: 67 - protein, 7 aa, synthetic construct
TRDTTYY

SEQ ID NO: 68 - protein, 6 aa, synthetic construct
DSAIYN

SEQ ID NO: 69 - protein, 6 aa, synthetic construct
VSGNPY

SEQ ID NO: 70 - protein, 6 aa, synthetic construct
YGGTVN

SEQ ID NO: 71 - protein, 6 aa, synthetic construct
SSVSVY

SEQ ID NO: 72 - protein, 7 aa, synthetic construct
TSESDYY

SEQ ID NO: 73 - protein, 5 aa, synthetic construct
KTLYG

SEQ ID NO: 74 - protein, 6 aa, synthetic construct
DSASNY

SEQ ID NO: 75 - protein, 6 aa, synthetic construct
TSGFNG

SEQ ID NO: 76 - protein, 6 aa, synthetic construct
SSNFYA

SEQ ID NO: 77 - protein, 6 aa, synthetic construct
DSASNY

SEQ ID NO: 78 - protein, 5 aa, synthetic construct
TTLSN

SEQ ID NO: 79 - protein, 5 aa, synthetic construct
SVFSS

SEQ ID NO: 80 - protein, 5 aa, synthetic construct
TTLSN

SEQ ID NO: 81 - protein, 6 aa, synthetic construct
NSASDY

SEQ ID NO: 82 - protein, 6 aa, synthetic construct
DSASNY

SEQ ID NO: 83 - protein, 6 aa, synthetic construct
DSAIYN

SEQ ID NO: 84 - protein, 6 aa, synthetic construct
TSGFYG

SEQ ID NO: 85 - protein, 6 aa, synthetic construct
NSAFQY

SEQ ID NO: 86 - protein, 5 aa, synthetic construct
SVFSS

SEQ ID NO: 87 - protein, 6 aa, synthetic construct
NSASQS

SEQ ID NO: 88 - protein, 6 aa, synthetic construct
DSAIYN

SEQ ID NO: 89 - protein, 6 aa, synthetic construct
YGATPY

SEQ ID NO: 90 - protein, 6 aa, synthetic construct
DSASNY

SEQ ID NO: 91 - protein, 7 aa, synthetic construct
VVTGGEV

SEQ ID NO: 92 - protein, 7 aa, synthetic construct
LYKAGEL

SEQ ID NO: 93 - protein, 8 aa, synthetic construct
QEAYKQQN

SEQ ID NO: 94 - protein, 8 aa, synthetic construct
QEAYKQQN

SEQ ID NO: 95 - protein, 7 aa, synthetic construct
LVKSGEV

SEQ ID NO: 96 - protein, 5 aa, synthetic construct
GLKNN

SEQ ID NO: 97 - protein, 8 aa, synthetic construct
RNSFDEQN

SEQ ID NO: 98 - protein, 7 aa, synthetic construct
IQSSQRE

SEQ ID NO: 99 - protein, 8 aa, synthetic construct
YITGDNLV

SEQ ID NO: 100 - protein, 8 aa, synthetic construct
YFSGDPLV

SEQ ID NO: 101 - protein, 8 aa, synthetic construct
YLSGSTLV

SEQ ID NO: 102 - protein, 8 aa, synthetic construct
QEAYKQQN

SEQ ID NO: 103 - protein, 7 aa, synthetic construct
LQKGGEE

SEQ ID NO: 104 - protein, 7 aa, synthetic construct
IRSNVGE

SEQ ID NO: 105 - protein, 6 aa, synthetic construct
NVLDGL

SEQ ID NO: 106 - protein, 7 aa, synthetic construct
MTLNGDE

SEQ ID NO: 107 - protein, 7 aa, synthetic construct
IRSNVGE

SEQ ID NO: 108 - protein, 7 aa, synthetic construct
LVKSGEV

SEQ ID NO: 109 - protein, 7 aa, synthetic construct
VVTGGEV

SEQ ID NO: 110 - protein, 7 aa, synthetic construct
LVKSGEV

SEQ ID NO: 111 - protein, 7 aa, synthetic construct
IRSNMDK

SEQ ID NO: 112 - protein, 7 aa, synthetic construct
IRSNVGE

SEQ ID NO: 113 - protein, 7 aa, synthetic construct
IQSSQRE

SEQ ID NO: 114 - protein, 6 aa, synthetic construct
NALDGL

SEQ ID NO: 115 - protein, 6 aa, synthetic construct
TYSSGN

SEQ ID NO: 116 - protein, 7 aa, synthetic construct
VVTGGEV

SEQ ID NO: 117 - protein, 6 aa, synthetic construct
VYSSGN

SEQ ID NO: 118 - protein, 7 aa, synthetic construct
IQSSQRE

SEQ ID NO: 119 - protein, 8 aa, synthetic construct
YFSGDTLV

SEQ ID NO: 120 - protein, 7 aa, synthetic construct
IRSNVGE

SEQ ID NO: 121 - protein, 12 aa, synthetic construct
AGDGSGNTGKLI

SEQ ID NO: 122 - protein, 17 aa, synthetic construct
AGAGGFLNSGGSKYKLT

SEQ ID NO: 123 - protein, 11 aa, synthetic construct
AFMKGSNYKLT

SEQ ID NO: 124 - protein, 12 aa, synthetic construct
ATHSGAGSYQLT

SEQ ID NO: 125 - protein, 11 aa, synthetic construct
AGNVGGTGKLI

SEQ ID NO: 126 - protein, 10 aa, synthetic construct
QRRDTGNQFY

SEQ ID NO: 127 - protein, 13 aa, synthetic construct
ALSEIKNQGGKLI

SEQ ID NO: 128 - protein, 8 aa, synthetic construct
AVRPGELS

SEQ ID NO: 129 - protein, 13 aa, synthetic construct
AVRDEGGATNKLI

SEQ ID NO: 130 - protein, 13 aa, synthetic construct
AVNAGGGSQGNLI

SEQ ID NO: 131 - protein, 10 aa, synthetic construct
AVSGSGDKLI

SEQ ID NO: 132 - protein, 11 aa, synthetic construct
ASFSGGYQKVT

SEQ ID NO: 133 - protein, 15 aa, synthetic construct
GAGRPNSGGSNYKLT

SEQ ID NO: 134 - protein, 10 aa, synthetic construct
AAGGRDDKII

SEQ ID NO: 135 - protein, 13 aa, synthetic construct
AVRPSNQAGTALI

SEQ ID NO: 136 - protein, 9 aa, synthetic construct
ASLYFNKFY

SEQ ID NO: 137 - protein, 4 aa, synthetic construct
AAIG

SEQ ID NO: 138 - protein, 11 aa, synthetic construct
AGAPSNDYKLS

SEQ ID NO: 139 - protein, 9 aa, synthetic construct
AGADNNDMR

SEQ ID NO: 140 - protein, 11 aa, synthetic construct
GTSNFGNEKLT

SEQ ID NO: 141 - protein, 13 aa, synthetic construct
AENDSGGGADGLT

SEQ ID NO: 142 - protein, 11 aa, synthetic construct
AAMRGGADGLT

SEQ ID NO: 143 - protein, 10 aa, synthetic construct
AVTGGADGLT

SEQ ID NO: 144 - protein, 8 aa, synthetic construct
ADQGGKLI

SEQ ID NO: 145 - protein, 10 aa, synthetic construct
AMKTSYDKVI

SEQ ID NO: 146 - protein, 11 aa, synthetic construct
AASGGSNYKLT

SEQ ID NO: 147 - protein, 12 aa, synthetic construct
AVNPSRGYSTLT

SEQ ID NO: 148 - protein, 9 aa, synthetic construct
AVYGNNRLA

SEQ ID NO: 149 - protein, 10 aa, synthetic construct
AVGYGNNRLA

SEQ ID NO: 150 - protein, 12 aa, synthetic construct
AAGPSNTGNQFY

SEQ ID NO: 151 - protein, 5 aa, synthetic construct
SEHNR

SEQ ID NO: 152 - protein, 5 aa, synthetic construct
LNHDA

SEQ ID NO: 153 - protein, 5 aa, synthetic construct
SEHNR

SEQ ID NO: 154 - protein, 5 aa, synthetic construct
SEHNR

SEQ ID NO: 155 - protein, 6 aa, synthetic construct
DFQATT

SEQ ID NO: 156 - protein, 5 aa, synthetic construct
SGHKS

SEQ ID NO: 157 - protein, 5 aa, synthetic construct
MGHRA

SEQ ID NO: 158 - protein, 5 aa, synthetic construct
MNHEY

SEQ ID NO: 159 - protein, 5 aa, synthetic construct
LNHDA

SEQ ID NO: 160 - protein, 5 aa, synthetic construct
MGHRA

SEQ ID NO: 161 - protein, 5 aa, synthetic construct
SEHNR

SEQ ID NO: 162 - protein, 5 aa, synthetic construct
MGHRA

SEQ ID NO: 163 - protein, 5 aa, synthetic construct
LGHNA

SEQ ID NO: 164 - protein, 5 aa, synthetic construct
MNHEY

SEQ ID NO: 165 - protein, 5 aa, synthetic construct
MGHRA

SEQ ID NO: 166 - protein, 5 aa, synthetic construct
MNHEY

SEQ ID NO: 167 - protein, 5 aa, synthetic construct
MNHEY

SEQ ID NO: 168 - protein, 6 aa, synthetic construct
DFQATT

SEQ ID NO: 169 - protein, 5 aa, synthetic construct
SGHTS

SEQ ID NO: 170 - protein, 5 aa, synthetic construct
SGHDT

SEQ ID NO: 171 - protein, 5 aa, synthetic construct
SGDLS

SEQ ID NO: 172 - protein, 5 aa, synthetic construct
SGHTA

SEQ ID NO: 173 - protein, 5 aa, synthetic construct
MNHEY

SEQ ID NO: 174 - protein, 5 aa, synthetic construct
MRHNA

SEQ ID NO: 175 - protein, 5 aa, synthetic construct
MGHDK

SEQ ID NO: 176 - protein, 5 aa, synthetic construct
MDHEN

SEQ ID NO: 177 - protein, 5 aa, synthetic construct
MNHEY

SEQ ID NO: 178 - protein, 5 aa, synthetic construct
KGHDR

SEQ ID NO: 179 - protein, 5 aa, synthetic construct
SGHRS

SEQ ID NO: 180 - protein, 5 aa, synthetic construct
MGHRA

SEQ ID NO: 181 - protein, 6 aa, synthetic construct
FQNEAQ

SEQ ID NO: 182 - protein, 6 aa, synthetic construct
SQIVND

SEQ ID NO: 183 - protein, 6 aa, synthetic construct
FQNEAQ

SEQ ID NO: 184 - protein, 6 aa, synthetic construct
FQNEAQ

SEQ ID NO: 185 - protein, 7 aa, synthetic construct
SNEGSKA

SEQ ID NO: 186 - protein, 6 aa, synthetic construct
YYEKEE

SEQ ID NO: 187 - protein, 6 aa, synthetic construct
YSYEKL

SEQ ID NO: 188 - protein, 6 aa, synthetic construct
SMNVEV

SEQ ID NO: 189 - protein, 6 aa, synthetic construct
SQIVND

SEQ ID NO: 190 - protein, 6 aa, synthetic construct
YSYEKL

SEQ ID NO: 191 - protein, 6 aa, synthetic construct
FQNEAQ

SEQ ID NO: 192 - protein, 6 aa, synthetic construct
YSYEKL

SEQ ID NO: 193 - protein, 6 aa, synthetic construct
YSLEER

SEQ ID NO: 194 - protein, 6 aa, synthetic construct
SMNVEV

SEQ ID NO: 195 - protein, 6 aa, synthetic construct
YSYEKL

SEQ ID NO: 196 - protein, 6 aa, synthetic construct
SMNVEV

SEQ ID NO: 197 - protein, 6 aa, synthetic construct
SVGEGT

SEQ ID NO: 198 - protein, 7 aa, synthetic construct
SNEGSKA

SEQ ID NO: 199 - protein, 6 aa, synthetic construct
YDEGEE

SEQ ID NO: 200 - protein, 6 aa, synthetic construct
YYEEEE

SEQ ID NO: 201 - protein, 6 aa, synthetic construct
YYNGEE

SEQ ID NO: 202 - protein, 6 aa, synthetic construct
FQGNSA

SEQ ID NO: 203 - protein, 6 aa, synthetic construct
SVGAGI

SEQ ID NO: 204 - protein, 6 aa, synthetic construct
SNTAGT

SEQ ID NO: 205 - protein, 6 aa, synthetic construct
SYGVNS

SEQ ID NO: 206 - protein, 6 aa, synthetic construct
SYDVKM

SEQ ID NO: 207 - protein, 6 aa, synthetic construct
SMNVEV

SEQ ID NO: 208 - protein, 6 aa, synthetic construct
SFDVKD

SEQ ID NO: 209 - protein, 6 aa, synthetic construct
YFSETQ

SEQ ID NO: 210 - protein, 6 aa, synthetic construct
YSYEKL

SEQ ID NO: 211 - protein, 21 aa, synthetic construct
ASSHNGLGQGEDLLSGANVLT

SEQ ID NO: 212 - protein, 11 aa, synthetic construct
ASSIPGGYGYT

SEQ ID NO: 213 - protein, 15 aa, synthetic construct
ASSPVNPAVSYNEQF

SEQ ID NO: 214 - protein, 11 aa, synthetic construct
ASSAPGYNEQF

SEQ ID NO: 215 - protein, 15 aa, synthetic construct
SARFIPTGLGENTIY

SEQ ID NO: 216 - protein, 13 aa, synthetic construct
ASSLTAGAYTGEL

SEQ ID NO: 217 - protein, 16 aa, synthetic construct
ASSQGVERQGPRNEQF

SEQ ID NO: 218 - protein, 12 aa, synthetic construct
ASSSSGRNNEQF

SEQ ID NO: 219 - protein, 11 aa, synthetic construct
ASSIAHGDEQY

SEQ ID NO: 220 - protein, 13 aa, synthetic construct
ASQDYLNSYNEQF

SEQ ID NO: 221 - protein, 15 aa, synthetic construct
ASSLARQGVDQETQY

SEQ ID NO: 222 - protein, 14 aa, synthetic construct
ASSQDKYRGNEKLF

SEQ ID NO: 223 - protein, 11 aa, synthetic construct
ASSQDRADTQY

SEQ ID NO: 224 - protein, 12 aa, synthetic construct
ASSLGGSRLEQY

SEQ ID NO: 225 - protein, 14 aa, synthetic construct
ASSPLDRGLSGELF

SEQ ID NO: 226 - protein, 14 aa, synthetic construct
ASSLSFGSGANVLT

SEQ ID NO: 227 - protein, 12 aa, synthetic construct
ASSYTSNTGELF

SEQ ID NO: 228 - protein, 12 aa, synthetic construct
SARGYGQGPEQY

SEQ ID NO: 229 - protein, 14 aa, synthetic construct
ASSPGTPFSYNEQF

SEQ ID NO: 230 - protein, 12 aa, synthetic construct
ASSFAVYGGELF

SEQ ID NO: 231 - protein, 13 aa, synthetic construct
ASSTLAGTYNEQF

SEQ ID NO: 232 - protein, 12 aa, synthetic construct
ASSLGPPGGEQF

SEQ ID NO: 233 - protein, 11 aa, synthetic construct
ASSYSNAGELF

SEQ ID NO: 234 - protein, 13 aa, synthetic construct
ASSLGLAGDDEQF

SEQ ID NO: 235 - protein, 9 aa, synthetic construct
ASSRGDEQF

SEQ ID NO: 236 - protein, 13 aa, synthetic construct
ASIGETGFVETQY

SEQ ID NO: 237 - protein, 12 aa, synthetic construct
ASSETGIRDGYT

SEQ ID NO: 238 - protein, 15 aa, synthetic construct
ATSDPSDRVGQETQY

SEQ ID NO: 239 - protein, 11 aa, synthetic construct
ASSLEGSREQY

SEQ ID NO: 240 - protein, 15 aa, synthetic construct
ASSLHIAGGISDTQY

SEQ ID NO: 241 - protein, 27 aa, synthetic construct
RAKRSGSGATNFSLLKQAGDVEENPGP

SEQ ID NO: 242 - protein, 19 aa, synthetic construct
ATNFSLLKQAGDVEENPGP

SEQ ID NO: 243 - protein, 141 aa, synthetic construct
NIQNPDPAVYQLRDSKSSDKSVCLFTDFDSQTNVSQSKDSDVYITDKTVLDMRSMDFKSNSAVAWSNKSDFACANAFNNSIIPEDTFFPSPESSCDVKLVEKSFETDTNLNFQNLSVIGFRILLLKVAGFNLLMTLRLWSS

SEQ ID NO: 244 - protein, 177 aa, synthetic construct
EDLKNVFPPEVAVFEPSEAEISHTQKATLVCLATGFFPDHVELSWWVNGKEVHSGVSTDPQPLKEQPALNDSRYCLSSRLRVSATFWQNPRNHFRCQVQFYGLSENDEWTQDRAKPVTQIVSAEAWGRADCGFTSVSYQQGVLSATILYEILLGKATLYAVLVSALVLMAMVKRKDF

SEQ ID NO: 245 - protein, 137 aa, synthetic construct
NIQNPEPAVYQLKDPRSQDSTLCLFTDFDSQINVPKTMESGTFITDKTVLDMKAMDSKSNGAIAWSNQTSFTCQDIFKETNTTYPSSDVPCDATLTEKSFETDMNLNFQNLSVMGLRILLLKVAGFNLLMTLRLWSS

SEQ ID NO: 246 - protein, 173 aa, synthetic construct
EDLRNVTPPKVSLFEPSKAEIANKQKATLVCLARGFFPDHVELSWWVNGKEVHSGVSTDPQAYKESNYSYCLSSRLRVSATFWHNPRNHFRCQVQFHGLSEEDKWPEGSPKPVTQNISAEAWGRADCGITSASYQQGVLSATILYEILLGKATLYAVLVSTLVVMAMVKRKNS

SEQ ID NO: 247 - protein, 141 aa, synthetic construct
XIQNPDPAVYQLRDSKSSDKSVCLFTDFDSQTNVSQSKDSDVYITDKCVLDMRSMDFKSNSAVAWSNKSDFACANAFNNSIIPEDTFFPSPESSCDVKLVEKSFETDTNLNFQNLSVIGFRILLLKVAGFNLLMTLRLWSS

SEQ ID NO: 248 - protein, 177 aa, synthetic construct
XDLKNVFPPEVAVFEPSEAEISHTQKATLVCLATGFFPDHVELSWWVNGKEVHSGVCTDPQPLKEQPALNDSRYCLSSRLRVSATFWQNPRNHFRCQVQFYGLSENDEWTQDRAKPVTQIVSAEAWGRADCGFTSVSYQQGVLSATILYEILLGKATLYAVLVSALVLMAMVKRKDF

SEQ ID NO: 249 - protein, 9 aa, synthetic construct
KVLEHVVRV

SEQ ID NO: 250 - protein, 10 aa, synthetic construct
GVYDGREHTV

SEQ ID NO: 251 - protein, 9 aa, synthetic construct
ALLEEEEGV

SEQ ID NO: 252 - protein, 9 aa, synthetic construct
KVDELAHFL

SEQ ID NO: 253 - protein, 10 aa, synthetic construct
ALAETSYVKV

SEQ ID NO: 254 - protein, 9 aa, synthetic construct
ALSNKVDEL

SEQ ID NO: 255 - protein, 9 aa, synthetic construct
GVAGDVSAV